European Patent Specification EP 3 946 391 B1, published March 25, 2026. Title: MICROBIAL CONSORTIUM AND USES THEREOF. Applicant: BIOMICA. The sequence listing filed with the application follows.

SEQUENCE LISTING (14 sequences)

SEQ ID NO: 1 - DNA, 1545 bp, Oenococcus oeni
agagtttgatcctggctcaggatgaacgctggtggcgtgcctaatacatgcaagtcgtacgctagccgctgaattgatccttcgggtgaagtgaggcaatgactagagtggcgaactggtgagtaacacgtaagaaacctgccctttagtgggggataacatttggaaacagatgctaataccgcgtaacaacaaatcacacatgtgatctgtttgaaaggtccttttggatcgctagaggatggtcttgcggcgtattagcttgttggtagggtagaagcctaccaaggcaatgatgcgtagccgagttgagagactggccggccacattgggactgagacactgcccaaactcctacgggaggctgcagtagggaattttccgcaatgcacgaaagtgtgacggagcgacgccgcgtgtgtgatgaaggctttcgggtcgtaaagcactgttgtaagggaagaataactgaattcagagaaagttttcagcttgacggtaccttaccagaaagggatggctaaatacgtgccagcagccgcggtaatacgtatgtcccgagcgttatccggatttattgggcgtaaagcgagcgcagacggtttattaagtctgatgtgaaatcccgaggcccaacctcggaactgcattggaaactgatttacttgagtgcgatagaggcaagtggaactccatgtgtagcggtgaaatgcgtagatatgtggaagaacaccagtggcgaaagcggcttgctagatcgtaactgacgttgaggctcgaaagtatgggtagcaaacgggattagataccccggtagtccataccgtaaacgatgggtgctagttgttaagaggtttccgcctcctagtgacgtagcaaacgcattaagcaccccgcctgaggagtacggccgcaaggctaaaacttaaaggaattgacggggacccgcacaagcggtggagcatgtggtttaattcgaagatacgcgaaaaaccttaccaggtcttgacataccaatgatcgcttttgtaatgaaagcttttcttcggaacattggatacaggtggtgcatggtcgtcgtcagctcgtgtcgtgagatgttgggttaagtcccgcaacgagcgcaacccttgttattagttgccagcatttagttgggcactctaatgagactgccggtgataaaccggaggaaggtggggacgacgtcagatcatcatgccccttatgacctgggcaacacacgtgctacaatgggaagtacaacgagtcgcaaaccggcgacggtaagctaatctcttaaaacttctctcagttcggactggagtctgcaactcgactccacgaaggcggaatcgctagtaatcgcgaatcagcatgtcgcggtgaatacgttcccgggtcttgtacacaccgcccgtcaaatcatgggagtcggaagtacccaaagtcgcttggctaacttttagaggccggtgcctaaggtaaaatcgatgactgggattaagtcgtaacaaggtagccgtaggagaacctgcggctgg

SEQ ID NO: 2 - DNA, 1456 bp, Clostridium tyrobutyricum
  misc_feature (518)..(518): n is a, c, g, or t
  misc_feature (939)..(940): n is a, c, g, or t
  misc_feature (1131)..(1131): n is a, c, g, or t
  misc_feature (1358)..(1358): n is a, c, g, or t
  misc_feature (1449)..(1449): n is a, c, g, or t
  misc_feature (1452)..(1452): n is a, c, g, or t
tttaaattgagagtttgatcctggctcaggacgaacgctggcggcgtgcctaacacatgcaagtcgagcgatgaaacccttcggggggggattagcggcggacgggtgagtaacacgtgggtaacctgcctcaaagtgggggatagccttccgaaaggaagattaataccgcataaagccaagtttcacatggaatttggatgaaaggagtaattcgctttgagatggacccgcggcgcattagttagttggtggggtaatggcctaccaagacagcgatgcgtagccgacctgagagggtgatcggccacattggaactgagatacggtccagactcctacgggaggcagcagtggggaatattgcacaatgggcgaaagcctgatgcagcaacgccgcgtgagtgatgaaggtcttcggattgtaaagctctgtcttttgggacgataatgacggtaccaaaggaggaagccacggctaactacgtgccagcagccgcggtaatacgtaggtggcnagcgttgtccggatttactgggcgtaaagggtgcgtaggcggatgtttaagtgagatgtgaaatacccgggcttaacttgggtgctgcatttcaaactggatatctagagtgcaggagaggagaatggaattcctagtgtagcggtgaaatgcgtagagattaggaagaacaccagtggcgaaggcgattctctggactgtaactgacgctgaggcacgaaagcgtgggtagcaaacaggattagataccctggtagtccacgccgtaaacgatgagtactaggtgtaggaggtatcgaccccttctgtgccgcagtaaacacattaagtactccgcctgggaagtacgatcgcaagattaaaactcaaaggaattgacgggggcccgcacaagcagcggagcatgtggtttaattcgaannaacgcgaagaaccttacctggacttgacatcccctgaataacctagagataggcgaacccttcggggcagggagacaggtggtgcatggttgtcgtcagctcgtgtcgtgagatgttaggttaagtcctgcaacgagcgcaacccttattgttagttgctaacattcagttgagcactctaacgagactgncgcggttaacgcggaggaaggtggggatgacgtcaaatcatcatgccccttatgtccagggcaacacacgtgctacaatgggcagaacaaagagaagcaataccgcgaggtggagccaaactcaaaaactgctctcagttcggattgcaggctgaaactcgcctgcatgaagctggagttgctagtaatcgcgaatcagcatgtcgcggtgaatacgttcccgggcnttgtacacaccgcccgtcacaccatgagagctggcaacacccgaagtccgtagtctaacgtaagaggacgcggccgaaggtggggttagtnatngggg

SEQ ID NO: 3 - DNA, 1470 bp, Cetobacterium somerae
agagtttgatcctggctcaggatgaacgctgacagaatgcttaacacatgcaagtcgattcgatttaccttcgggtattgaggatggcggacgggtgagtaacgcgtaaggaacttgcctcttggtctgggacaactgttggaaacgacagctaataccggatattatgagattctcgcatgggaaacttatgaaagctatatgcgccaagagagagccttgcgttccattagctagttggtggggtaacggcccaccaaggcgacgatggatagccggcctgagagggtgaacggccacaaggggactgagacacggcccttactcctacgggaggcagcagtggggaatattggacaatgggccacaagcctgatccagcaattctgtgtgcacgatgaaggtcttcggattgtaaagtgctttcagttgggaagaagaaagtgacggtaccaacagaagaagcgacggctaaatacgtgccagcagccgcggtaatacgtatgtcgcaagcgttatccggatttattgggcgtaaagcgcgtctaggcggaaaaataagtctgatgttaaaatgcggggctcaactccgtattgcgttggaaactgtttttctagagtactggagaggtgggcggaactacaagtgtagaggtgaaattcgtagatatttgtaggaatgccgatggagaagtcagctcactggacagatactgacgctaaagcgcgaaagcgtggggagcaaacaggattagataccctggtagtccacgccgtaaacgatgatcactaggtgttgggggtcgaacctcagcgcccaagctaacgcgataagtgatccgcctggggagtacgcacgcaagtgtgaaactcaaaggaattgacggggacccgcacaagcggtggagcatgtggtttaattcgacgcaacgcgagaaaccttaccagcgtttgacatcctaagaagtttccagagatggattcgtgccggcttgccggaacttagtgacaggtggtgcatggctgtcgtcagctcgtgtcgtgagatgttgggttaagtcccgcaacgagcgcaacccctattgtatgttgctaccattaagttgagcactcatgcgatactgcctgcgatgagcaggaggaaggtggggatgacgtcaagtcatcatgccccttatacgctgggctacacacgtgctacaatgggcagtacagagagttgccaacccgcgagggtgagctaatctcttaaagctgttcttagttcggattgtactctgcaactcgagtacatgaagttggaatcgctagtaatcgcaaatcagcatgttgcggtgaatacgttctcgggtcttgtacacaccgcccgtcacaccacgagagttggttgcacctgaagtagcaggcctaaccgtaaggagggatgttcctaaggtgtgattagcgattggggtgaagtcgtaacaaggt

SEQ ID NO: 4 - DNA, 1516 bp, Corynebacterium glyciniphilum
agagtttgatcctggctcaggacgaacgctggcggcgtgcttaacacatgcaagtcgaacggaaaggccctgcttgcagggtactcgagtggcgaacgggtgagtaacacgtgggtgatctgccctgcacttcgggataagcctgggaaactgggtctaataccggataggaccatcgtttagtgtcggtggtggaaagtttttcggtgcaggatgagcccgcggcctatcagcttgttggtggggtaatggcctaccaaggcgtcgacgggtagccggcctgagagggtggacggccacattgggactgagacacggcccagactcctacgggaggcagcagtggggaatattgcacaatgggcgcaagcctgatgcagcgacgccgcgtgggggatgaaggccttcgggttgtaaactcctttcagccatgacgaagctggccttgttgggtcagtgacggtagtggtagaagaagcaccggctaactacgtgccagcagccgcggtaatacgtagggtgcgagcgttgtccggaattactgggcgtaaagagctcgtaggtggtttgtcacgtcgtctgtgaaattccggggcttaactccgggcgtgcaggcgatacgggcataacttgagtactgtaggggagactggaattcctggtgtagcggtgaaatgcgcagatatcaggaggaacaccgatggcgaaggcaggtctctgggcagttactgacgctgaggagcgaaagcatgggtagcgaacaggattagataccctggtagtccatgccgtaaacggtgggcgctaggtgtgggggtcttccacgacttccgtgccgtagctaacgcattaagcgccccgcctggggagtacggccgcaaggctaaaactcaaaggaattgacgggggcccgcacaagcggcggagcatgtggattaattcgatgcaacgcgaagaaccttacctgggcttgacatatgcaggatcggcacagagatgtgttttcccttgtggtctgtatacaggtggtgcatggttgtcgtcagctcgtgtcgtgagatgttgggttaagtcccgcaacgagcgcaacccttgtcttgtgttgccagcacgttatggtggggactcgcgagagactgccggggttaactcggaggaaggtggggatgacgtcaaatcatcatgccccttatgtccagggcttcacacatgctacaatggtcggtacagtgggttgcgataccgtgaggtggagctaatcccttaaagccggtctcagttcggattggagtctgcaactcgactccatgaagtcggagtcgctagtaatcgcagatcagcaacgctgcggtgaatacgttcccgggccttgtacacaccgcccgtcacgtcatgaaagttggtaacacccgaagccagtggcccaaactcgttagggagctgtcgaaggtgggatcggcgattgggacgaagtcgtaacaaggtagccgtaccggaaggtgcggctggatcacct

SEQ ID NO: 5 - DNA, 1506 bp, Clostridium cellulovorans
gagagtttgatcctggctcaggacgaacgctggcggcgtgcttaacacatgcaagtcgagcgatgaagcttcggggtggattagcggcggacgggtgagtaacacgtgggcaacctgccttatagagggggatagccttccgaaaggaagattaataccgcataaaatgcaattctcgcatgagagatgtatcaaaggagcaatccgctataagatgggcccgcggcgcattagctagttggttaggtaacgactcaccaaggcgacgatgcgtagccgacctgagagggtgatcggccacattggaactgagacacggtccagactcctacgggaggcagcagtggggaatattgcacaatgggggaaaccctgatgcagcaacgccgcgtgagtgatgaaggccttcgggttgtaaagctctttgattagggacgataatgacggtacctaaagaacaagccacggctaactacgtgccagcagccgcggtaatacgtaggtggcaagcgttgtccggatttactgggcgtaaaggatgtgtaggcggatttttaagtgagatgtgaaatacccgagctcaacttgggtgctgcatttcaaactggaagtctagagtgcaggagaggaaagtggaattcctagtgtagcggtgaaatgcgtagagattaggaagaacatcagtggcgaaggcgactttctggactgtaactgacgctgaggcatgaaagcgtggggagctaaacaggattagataccctggtagtccacgccgtaaacgatgaatactaggtgtaggggttgtcatgacctctgtgccgcccgctaacgcattaagtattccgcctggggagtacggtcgcaagattaaaactcaaaggaattgacgggggcccgcacaagcagcggacgatgtggtttaattcgaagcaacgcgaagaaccttacctagacttgacatctcctgaattacccgtaactggggaagttacctctttgaggtgacaggaagacaggtggtgcatggttgtcgtcagctcgtgtcgtcagatgttgggttaagtcccgcaacgagcgcaacccttattgttagttgctaccatttagttgagcactctagcaagactgcctgggttaaccaggaggaaggtggggatgacgtccaatcatcatgccccttatgtctagggctacacacgtgctacaatggcgagtacaacgagacgcaagaccgtgaggtggagcaaatctataaaactcgtcccagttcggattgtaggctgaaactcgcctacatgaagttggagttgctagtaatcgcgaatcagcatgtcgcggtgaatacgttcccgggccttgtacacaccgcccgtcacaccatgagagtcggcaacacccgaagtccgtgaggtaaccgtaaggagccagcggccgaaggtggggtcgatgattggggtgaagtcgtaacaaggtagcgtagagaacctgcggttggatcacctcctt

SEQ ID NO: 6 - DNA, 1425 bp, Methanosphaera stadtmanae
  misc_feature (590)..(590): n is a, c, g, or t
  misc_feature (894)..(896): n is a, c, g, or t
aatccgtttgatcctggcggaagctactgctattgggattcgattaagccatgcaagtcgaatgaacctagttcatggcatacggctcagtaacacgtggataacctacccttaggaccgggataactttgggaaactgaagataatactggatattaggttatgcctggaatggtttacctttgaaatgtatttttcgcctaaggatagatctgcggctgattaggtcgttggtggggtaatggcccaccaagccgatgatcggtacgggttgtgagagcaagagcccggagatggaacctgagacaaggttccagaccctacggggtgcagcaggcgcgaaacctccgcaatgtacgcaagtgcgacggggggatcccaagtgttattcttaacagaataacttttcattagtgtaaaaagcttttagaataagagctgggcaagaccggtgccagccgccgcggtaacaccggcagctcaagtggtagctgtttttattgggcctaaagcgttcgtagccggtttgataagtctttggtgaaagcttgtagcttaactataagaattgctgaagatactgtcagacntgaagtcgggagaggttagaggtactaccggggtaggggtgaaatcctataatcctgggaggaccacctgtggcgaaggcgtctaactggaacgatcttgacggtgagtaacgaaagccaggggcgcgaaccggattagatacccgggtagtcctggccgtaaacgatgtggacttggtgttggaatggcctcgagttgttccggtgccgaagggaagctgttaagtccaccgcctgggaagtacggtcgcaagactgaaacttaaaggaattggcgggggagcaccacaacgcgtggagcctnnngtttaattggattcaacgccggacatctcaccaggagcgacagcagaatgataatcaggttgatgaccttatttgactagctgagaggaggtgcatggccgccgtcagctcgtaccgtgaagcgtcctgttaagtcaggcaacgagcgagacccacgcccttagttaccaacacaatctctggattggtgggcacactagggggaccgccagtgataaactggaggaaggagtggacgacggtaggtcagtatgccccgaatctcctgggctacacgcgggctacaatggctatggcaatgggtttctgcactgaaaagtgatggtaatctcctaaacatagtcttagttcggattgagggctgtaactcgccctcatgaagctggaatgcgtagtaatcgcatgtcacaaccgtgcggtgaatacgtccctgctccttgcacacaccgcccgtcacaccacccaaaaagggtttggatgaggccataattttcaaatgttattgtcgaatctaggttttttgaggagg

SEQ ID NO: 7 - DNA, 1500 bp, Veillonella parvula
gcgaagctggcggcgtgcttaacacatgcaagtcgaacgaagagcgatggaagcttgcttctatcaatcttagtggcgaacgggtgagtaacgcgtaatcaacctgcccttcagagggggacaacagttggaaacgactgctaataccgcatacgatctaatctcggcatcgaggatagatgaaaggtggcctctacatgtaagctatcactgaaggaggggattgcgtctgattagctagttggaggggtaacggcccaccaaggcgatgatcagtagccggtctgagaggatgaacggccacattgggactgagacacggcccagactcctacgggaggcagcagtggggaatcttccgcaatggacgaaagtctgacggagcaacgccgcgtgagtgatgacggccttcgggttgtaaagctctgttaatcgggacgaaaggccttcttgcgaatagtgagaaggattgacggtaccggaatagaaagccacggctaactacgtgccagcagccgcggtaatacgtaggtggcaagcgttgtccggaattattgggcgtaaagcgcgcgcaggcggatmggtcagtctgtcttaaaagttcggggcttaaccccgtgatgggatggaaactgccaatctagagtatcggagaggaaagtggaattcctagtgtagcggtgaaatgcgtagatattaggaagaacaccagtggcgaaggcgactttctggacgaaaactgacgctgaggcgcgaaagccaggggagcgaacgggattagataccccggtagtcctggccgtaaacgatgggtactaggtgtaggaggtatcgaccccttctgtgccggagttaacgcaataagtaccccgcctggggagtacgaccgcaaggttgaaactcaaaggaattgacgggggcccgcacaagcggtggagtatgtggtttaattcgacgcaacgcgaagaaccttaccaggtcttgacattgatggacagaaccagagatggttcctcttcttcggaagccagaaaacaggtggtgcacggttgtcgtcagctcgtgtcgtgagatgttgggttaagtcccgcaacgagcgcaacccctatcttatgttgccagcactttgggtggggactcatgagagactgccgcagacaatgcggaggaaggcggggatgacgtcaaatcatcatgccccttatgacctgggctacacacgtactacaatgggagttaatagacggaagcgagatcgcgagatggagcaaacccgagaaacactctctcagttcggatcgtaggctgcaactcgcctacgtgaagtcggaatcgctagtaatcgcaggtcagcatactgcggtgaatacgttcccgggccttgtacacaccgcccgtcacaccacgaaagtcggaagtgcccaaagccggtggggtaaccttcgggagccagccgtctaaggtaaagtcgatgattggggtgaagtcgtaacaaggtag

SEQ ID NO: 8 - DNA, 1509 bp, Bacteroides caccae
agagtttgatcctggctcaggatgaacgctagctacaggcttaacacatgcaagtcgaggggcatcagtttggtttgcttgcaaaccaaagctggcgaccggcgcacgggtgagtaacacgtatccaacctgcctcatactcggggatagcctttcgaaagaaagattaatatccgatagcatatatttcccgcatgggttttatattaaagaaattcggtatgagatggggatgcgttccattagtttgttgggggggtaacggcccaccaagactacgatggataggggttctgagaggaaggtcccccacattggaactgagacacggtccaaactcctacgggaggcagcagtgaggaatattggtcaatggacgcgagtctgaaccagccaagtagcgtgaaggatgactgccctatgggttgtaaacttcttttatatgggaataaagttgtccacgtgtggatttttgtatgtaccatatgaataaggatcggctaactccgtgccagcagccgcggtaatacggaggatccgagcgttatccggatttattgggtttaaagggagcgtaggcggattgttaagtcagttgtgaaagtttgcggctcaaccgtaaaattgcagttgatactggcagtcttgagtgcagtagaggtgggcggaattcgtggtgtagcggtgaaatgcttagatatcacgaagaactccgattgcgaaggcagctcactggagtgtaactgacgctgatgctcgaaagtgtgggtatcaaacaggattagataccctggtagtccacacagtaaacgatgaatactcgctgtttgcgatatacagtaagcggccaagcgaaagcattaagtattccacctggggagtacgccggcaacggtgaaactcaaaggaattgacgggggcccgcacaagcggaggaacatgtggtttaattcgatgatacgcgaggaaccttacccgggcttaaattgcaaatgaattatggggaaacccatacgccgcaaggcatttgtgaaggtgctgcatggttgtcgtcagctcgtgccgtgaggtgtcggcttaagtgccataacgagcgcaacccttatcttcagttactaacaggtcatgctgaggactctggagagactgccgtcgtaagatgtgaggaaggtggggatgacgtcaaatcagcacggcccttacgtccggggctacacacgtgttacaatggggggtacagaaggccgctacctggtgacaggatgccaatcccaaaaacctctctcagttcggatcgaagtctgcaacccgacttcgtgaagctggattcgctagtaatcgcgcatcagccatggcgcggtgaatacgttcccgggccttgtacacaccgcccgtcaagccatgaaagccgggggtacctgaagtacgtaaccgcaaggagcgtcctagggtaaaactggtaattggggctaagtcgtaacaaggtagccgtaccggaaggtgcggctg

SEQ ID NO: 9 - DNA, 1559 bp, Lactobacillus casei
tttgatcatggctcaggatgaacgctggcggcgtgcctaatacatgcaagtcgaacgagttctcgttgatgatcggtgcttgcaccgagattcaacatggaacgagtggcggacgggtgagtaacacgtgggtaacctgcccttaagtgggggataacatttggaaacagatgctaataccgcatagatccaagaaccgcatggttcttggctgaaagatggcgtaagctatcgcttttggatggacccgcggcgtattagctagttggtgaggtaatggctcaccaaggcgatgatacgtagccgaactgagaggttgatcggccacattgggactgagacacggcccaaactcctacgggaggcagcagtagggaatcttccacaatggacgcaagtctgatggagcaacgccgcgtgagtgaagaaggctttcgggtcgtaaaactctgttgttggagaagaatggtcggcagagtaactgttgtcggcgtgacggtatccaaccagaaagccacggctaactacgtgccagcagccgcggtaatacgtaggtggcaagcgttatccggatttattgggcgtaaagcgagcgcaggcggttttttaagtctgatgtgaaagccctcggcttaaccgaggaagcgcatcggaaactgggaaacttgagtgcagaagaggacagtggaactccatgtgtagcggtgaaatgcgtagatatatggaagaacaccagtggcgaaggcggctgtctggtctgtaactgacgctgaggctcgaaagcatgggtagcgaacaggattagataccctggtagtccatgccgtaaacgatgaatgctaggtgttggagggtttccgcccttcagtgccgcagctaacgcattaagcattccgcctggggagtacgaccgcaaggttgaaactcaaaggaattgacgggggcccgcacaagcggtggagcatgtggtttaattcgaagcaacgcgaagaaccttaccaggtcttgacatcttttgatcacctgagagatcaggtttccccttcgggggcaaaatgacaggtggtgcatggttgtcgtcagctcgtgtcgtgagatgttgggttaagtcccgcaacgagcgcaacccttatgactagttgccagcatttagttgggcactctagtaagactgccggtgacaaaccggaggaaggtggggatgacgtcaaatcatcatgccccttatgacctgggctacacacgtgctacaatggatggtacaacgagttgcgagaccgcgaggtcaagctaatctcttaaagccattctcagttcggactgtaggctgcaactcgcctacacgaagtcggaatcgctagtaatcgcggatcagcacgccgcggtgaatacgttcccgggccttgtacacaccgcccgtcacaccatgagagtttgtaacacccgaagccggtggcgtaacccttttagggagcgagccgtctaaggtgggacaaatgattagggtgaagtcgtaacaaggtagccgtaggagaacctgcggctggatcacctcctta

SEQ ID NO: 10 - DNA, 1407 bp, Ruminococcus albus
ttgatcctggctcaggacgaacgctggcggcacgcttaacacatgcaagtcgaacgagcgaaagagtgcttgcactctctagctagtggcgggcgggtgagtaacacgtgagcaatctgcctttcggagagggataccaattggaaacgattgttaatacctcataacataacgaagccgcatgactttgttatcaaatgaatttcgccgaaagatgagctcgcgtctgattaggtagttggtgaggtaacggcccaccaagccgacgatcagtagccggactgagaggttgaacggccacattgggactgagacacggcccagactcctacgggaggcagcagtggggaatattgcacaatgggcgaaagcctgatgcagcgatgccgcgtgagggaagaaggttttaggattgtaaacctctgtctttggggacgataatgacggtacccaaggaggaagctccggctaactacgtgccagcagccgcggtaatacgtagggagcgagcgttgtccggaattactgggtgtaaagggagcgtaggcgggattgcaagtcaggtgtgaaatttaggggcttaacccctgaactgcacttgaaactgtagttcttgagtgaagtagaggtaagcggaattcctagtgtagcggtgaaatgcgtagatattaggaggaacatcagtggcgaaggcggcttactgggctttaactgacgctgaggctcgaaagcgtggggagcaaacaggattagataccctggtagtccacgccgtaaacgatgattactaggtgtggggggactgaccccttccgtgccgcagttaacacaataagtaatccacctggggagtacggccgcaaggctgaaactcaaaggaattgacgggggcccgcacaagcagtggagtatgtggtttaattcgaagcaacgcgaagaaccttaccaggtcttgacatcgtacgcatagcatagagatatgtgaaatcccttcggggacgtatagacaggtggtgcatggttgtcgtcagctcgtgtcgtgagatgttgggttaagtcccgcaacgagcgcaacccttactgttagttgctacgcaagagcactctagcaggactgccgttgacaaaacggaggaaggtggggatgacgtcaaatcatcatgccccttatgacctgggctacacacgtactacaatggctgttaacagagggaagcaaaacagtgatgtggagcaaaaccctaaaagcagtcttagttcggattgtaggctgcaacccgcctacatgaagtaggaattgctagtaatcgcggatcagcatgccgcggtgaatacgttcccgggccttgtacacaccgcccgtcacgccatgggagtcggtaaccccgaagcctgtgttctaaccgc

SEQ ID NO: 11 - DNA, 1520 bp, Bifidobacterium breve
ttcgattctggctcaggatgaacgctggcggcgtgcttaacacatgcaagtcgaacgggatccatcgggctttgcttggtggtgagagtggcgaacgggtgagtaatgcgtgaccgacctgccccatgcaccggaatagctcctggaaacgggtggtaatgccggatgctccatcacaccgcatggtgtgttgggaaagcctttgcggcatgggatggggtcgcgtcctatcagcttgatggcggggtaacggcccaccatggcttcgacgggtagccggcctgagagggcgaccggccacattgggactgagatacggcccagactcctacgggaggcagcagtggggaatattgcacaatgggcgcaagcctgatgcagcgacgccgcgtgagggatggaggccttcgggttgtaaacctcttttgttagggagcaaggcactttgtgttgagtgtacctttcgaataagcaccggctaactacgtgccagcagccgcggtaatacgtagggtgcaagcgttatccggaattattgggcgtaaagggctcgtaggcggttcgtcgcgtccggtgtgaaagtccatcgcttaacggtggatccgcgccgggtacgggcgggcttgagtgcggtaggggagactggaattcccggtgtaacggtggaatgtgtagatatcgggaagaacaccaatggcgaaggcaggtctctgggccgttactgacgctgaggagcgaaagcgtggggagcgaacaggattagataccctggtagtccacgccgtaaacggtggatgctggatgtggggcccgttccacgggttccgtgtcggagctaacgcgttaagcatcccgcctggggagtacggccgcaaggctaaaactcaaagaaattgacgggggcccgcacaagcggcggagcatgcggattaattcgatgcaacgcgaagaaccttacctgggcttgacatgttcccgacgatcccagagatggggtttcccttcggggcgggttcacaggtggtgcatggtcgtcgtcagctcgtgtcgtgagatgttgggttaagtcccgcaacgagcgcaaccctcgccccgtgttgccagcggattgtgccgggaactcacgggggaccgccggggttaactcggaggaaggtggggatgacgtcagatcatcatgccccttacgtccagggcttcacgcatgctacaatggccggtacaacgggatgcgacagtgcgagctggagcggatccctgaaaaccggtctcagttcggatcgcagtctgcaactcgactgcgtgaaggcggagtcgctagtaatcgcgaatcagcaacgtcgcggtgaatgcgttcccgggccttgtacacaccgcccgtcaagtcatgaaagtgggcagcacccgaagccggtggcctaaccccttgcgggagggagccgtctaaggtgaggctcgtgattgggactaagtcgtaacaaggtagccgtaccggaaggtgcggctggatcacctcctta

SEQ ID NO: 12 - DNA, 1468 bp, Alistipes putredini
  misc_feature (2)..(2): n is a, c, g, or t
  misc_feature (30)..(30): n is a, c, g, or t
  misc_feature (202)..(202): n is a, c, g, or t
  misc_feature (339)..(339): n is a, c, g, or t
  misc_feature (425)..(425): n is a, c, g, or t
  misc_feature (439)..(439): n is a, c, g, or t
  misc_feature (527)..(527): n is a, c, g, or t
  misc_feature (530)..(530): n is a, c, g, or t
  misc_feature (544)..(544): n is a, c, g, or t
  misc_feature (637)..(637): n is a, c, g, or t
  misc_feature (739)..(739): n is a, c, g, or t
  misc_feature (761)..(763): n is a, c, g, or t
  misc_feature (771)..(771): n is a, c, g, or t
  misc_feature (867)..(867): n is a, c, g, or t
  misc_feature (1127)..(1127): n is a, c, g, or t
  misc_feature (1139)..(1139): n is a, c, g, or t
  misc_feature (1204)..(1204): n is a, c, g, or t
  misc_feature (1425)..(1425): n is a, c, g, or t
cnatggagagtttgatcctggctcaggatnaacgctagcggcaggcttaacacatgcaagtcgaggggcagcatcatggatagcaatatctatggtcggcgaccggcgcacgggtgcgtaacgcgtatgcaacctacctttaacagggggataacaccgagaaattggtactaataccccataatatcatagaaggcatctnttatggttgaaaattccgatggttagagatgggcatgcgttgtattagctagttggtggggtaacggctcaccaaggcaacgatacatagggggactgagaggttaaccccccacactggtactgagacacggaccngactcctacgggaggcagcagtgaggaatattggtcaatggacgcaagtctgaaccagccatgccgcgtgcaggatgacggctctntgagttgtaaactncttttgtacgagggtaaacgcagatacgtgtatctgtctgaaagtatcgtacgaataaggatcggctaactccgtgccagcagccgcngtnatacggaggattcnagcgttatccggatttattgggtttaaagggtgcgtaggcggtttgataagttagaggtgaaatttcggggctcaaccctgaacgtgcctctnatactgttgagctagagagtagttgcggtaggcggaatgtatggtgtagcggtgaaatgcttagagatcatacagaacaccgattgcgaaggcagcttaccnaactatatctgacgctgatgcnnnaaagcgtngggagcaaacaggattagataccctggtagtccacgcagtaaacgatgataactcgttgtcggcgatacacagtcggtgactaagcgaaagcgatnagttatccacctggggagtacgttcgcaagaatgaaactcaaaggaattgacgggggcccgcacaagcggaggaacatgtggtttaattcgatgatacgcgaggaaccttacccgggcttgaaagttagcgacgattcttgaaagaggatttccttcggggcgcgaaactaggtgctgcatggttgtcgtcagctcgtgccgtgaggtgtcgggttaagtcccataacgagcgcaacccctaccgttagttgccatcagntgaagctgggcnctctggcgggactgccggtgtaagccgagaggaaggtggggatgacgtcaaatcagcacggcccntacgtccggggctacacacgtgttacaatggtaggtacagagggcagctacccagcgatgggatgcgaatctcgaaagcctatctcagttcggattggaggctgaaacccgcctccatgaagttggattcgctagtaatcgcgcatcagccatggcgcggtgaatacgttcccgggccttgtacacaccgcccgtcaagccatgggagccgggggtgcctnaagttcgtgaccgcaaggagcgacctagggcaaaactggtgac

SEQ ID NO: 13 - DNA, 1433 bp, Akkermansia muciniphila
aacgaacgctggcggcgtggataagacatgcaagtcgaacgagagaattgctagcttgctaataattctctagtggcgcacgggtgagtaacacgtgagtaacctgcccccgagagcgggatagccctgggaaactgggattaataccgcatagtatcgaaagattaaagcagcaatgcgcttggggatgggctcgcggcctattagttagttggtgaggtaacggctcaccaaggcgatgacgggtagccggtctgagaggatgtccggccacactggaactgagacacggtccagacacctacgggtggcagcagtcgagaatcattcacaatgggggaaaccctgatggtgcgacgccgcgtgggggaatgaaggtcttcggattgtaaacccctgtcatgtgggagcaaattaaaaagatagtaccacaagaggaagagacggctaactctgtgccagcagccgcggtaatacagaggtctcaagcgttgttcggaatcactgggcgtaaagcgtgcgtaggctgtttcgtaagtcgtgtgtgaaaggcgcgggctcaacccgcggacggcacatgatactgcgagactagagtaatggagggggaaccggaattctcggtgtagcagtgaaatgcgtagatatcgagaggaacactcgtggcgaaggcgggttcctggacattaactgacgctgaggcacgaaggccaggggagcgaaagggattagatacccctgtagtcctggcagtaaacggtgcacgcttggtgtgcggggaatcgaccccctgcgtgccggagtaacgcgttaagcgtgccgcctggggagtacggtcgcaagattaaaactcaaagaaattgacggggacccgcacaagcggtggagtatgtggcttaattcgatgcaacgcgaagaaccttacctgggcttgacatgtaatgaacaacatgtgaaagcatgcgactcttcggaggcgttacacaggtgctgcatggccgtcgtcagctcgtgtcgtgagatgtttggttaagtccagcaacgagcgcaacccctgttgccagttaccagcacgtgaaggtggggactctggcgagactgcccagatcaactgggaggaaggtggggacgacgtcaggtcagtatggcccttatgcccagggctgcacacgtactacaatgcccagtacagagggggccgaagccgcgaggcggaggaaatcctaaaaactgggcccagttcggactgtaggctgcaacccgcctacacgaagccggaatcgctagtaatggcgcatcagctacggcgccgtgaatacgttcccgggtcttgtacacaccgcccgtcacatcatggaagctggtcgcacccgaagtatctgaagccaaccgcaaggaggcagggtcctaaggtgagactggtaactgggatg

SEQ ID NO: 14 - DNA, 1516 bp, Akkermansia muciniphila
atggagagtttgattctggctcagaacgaacgctggcggcgtggataagacatgcaagtcgaacgggagaattgctagcttgctaataattctctagtggcgcacgggtgagtaacacgtgagtaacctgcccccgagagcgggatagccctgggaaactgggattaataccgcatagtatcgaaagattaaagcagcaatgcgcttggggatgggctcgcggcctattagttagttggtgaggtaacggctcaccaaggcgatgacgggtagccggtctgagaggatgtccggccacactggaactgagacacggtccagacacctacgggtggcagcagtcgagaatcattcacaatgggggaaaccctgatggtgcgacgccgcgtgggggaatgaaggtcttcggattgtaaacccctgtcatgtgggagcaaattaaaaagatagtaccacaagaggaagagacggctaactctgtgccagcagccgcggtaatacagaggtctcaagcgttgttcggaatcactgggcgtaaagcgtgcgtaggctgtttcgtaagtcgtgtgtgaaaggcgcgggctcaacccgcggacggcacatgatactgcgagactagagtaatggagggggaaccggaattctcggtgtagcagtgaaatgcgtagatatcgagaggaacactcgtggcgaaggcgggttcctggacattaactgacgctgaggcacgaaggccaggggagcgaaagggattagatacccctgtagtcctggcagtaaacggtgcacgcttggtgtgcggggaatcgaccccctgcgtgccggagctaacgcgttaagcgtgccgcctggggagtacggtcgcaagattaaaactcaaagaaattgacggggacccgcacaagcggtggagtatgtggcttaattcgatgcaacgcgaagaaccttacctgggcttgacatgtaatgaacaacatgtgaaagcatgcgactcttcggaggcgttacacaggtgctgcatggccgtcgtcagctcgtgtcgtgagatgtttggttaagtccagcaacgagcgcaacccctgttgccagttaccagcacgtgaaggtggggactctggcgagactgcccagatcaactgggaggaaggtggggacgacgtcaggtcagtatggcccttatgcccagggctgcacacgtactacaatgcccagtacagagggggccgaagccgcgaggcggagggaatcctaaaaactgggcccagttcggactgtaggctgcaacccgcctacacgaagccggaatcgctagtaatggcgcatcagctacggcgccgtgaatacgttcccgggtcttgtacacaccgcccgtcacatcatggaagccggtcgcacccgaagtatctgaagccaaccgcaaggaggcagggtcctaaggtgagactggtaactgggatgaagtcgtaacaaggtagccgtaggggaacctgcggctggatcacctcctttctatgga